European Patent Specification EP 3 442 352 B1, published June 3, 2026. Title: COMPOUNDS THAT MODULATE CALCIUM-SENSING RECEPTOR ACTIVITY FOR MODULATING KOKUMI TASTE AND PET FOOD PRODUCTS CONTAINING THE SAME. Applicant: MARS, INCORPORATED. The sequence listing filed with the application follows.

SEQUENCE LISTING (2 sequences)

SEQ ID NO: 1 - protein, 1081 aa, Felis catus
MAFYSCCLILLAITWCTSAYGPDQRAQKKGDIILGGLFPIHFGVAAKDQDLKSRPESVECIRYNFRGFRWLQAMIFAIEEINSSPVLLPNMTLGYRIFDTCNTVSKALEATLSFVAQNKIDSLNLDEFCNCSEHIPSTIAVVGATGSGISTAVANLLGLFYIPQVSYASSSRLLSNKNQFKSFLRTIPNDEHQATAMADIIEYFRWNWVGTIAADDDYGRPGIEKFREEAEERDICIDFSELISQYSDEEEIQQVVEVIQNSTAKVIVVFSSGPDLEPLIKEIVRRNITGRIWLASEAWASSSLIAMPEYFHVVGGTIGFALKAGQIPGFREFLQKVHPRKSVHNGFAKEFWEETFNCHLQEGAKGPLALDTFLRGHEEGGGRISNSSTALRPLCTGDENISSVETPYMDYTHLRISYNVYLAVYSIAHALQDIYTCLPGRGLFTNGSCADIKKVEAWQVLKHLRHLNFTNNMGEQVTFDECGDLVGNYSIINWHLSPEDGSIVFKEVGYYNVYAKKGERLFINEEKILWSGFSREVPFSNCSRDCLAGTRKGIIEGEPTCCFECVECPDGEYSDETDASACDKCPDDFWSNENHTSCIAKEIEFLSWTEPFGIALTLFAVLGIFLTAFVLGVFLKFRNTPIVKATNRELSYLLLFSLLCCFSSSLFFIGEPQDWTCRLRQPAFGISFVLCISCILVKTNRVLLVFEAKIPTSFHRKWWGLNLQFLLVFLCTFMQIVICVIWLYTAPPSSYRNHELEDEIIFITCHEGSLMALGFLIGYTCLLAAICFFFAFKSRKLPENFNEAKFITFSMLIFFIVWISFIPAYASTYGKFVSAVEVIAILAASFGLLACIFFNKVYIILFKPSRNTIEEVRCSTAAHAFKVAARATLRRSNVSRKRSSSLGGSTGSTPSSSISSKSNSEDPFPQPERQKQQQPLALTQQEQQPQPQQPSSLQQQPQPQPQPRCKQKVIFGSGTVTFSLSFDEPQKSAMAHRNSMHQNSLEAQKSNETLTRHQALLPLQCGETDSELSAQERGLQGPVDGDFRPEMEDPEEMSPALVVSSSQSFVISGGGSTVTENILHS

SEQ ID NO: 2 - DNA, 3243 bp, Felis catus
atggcattttatagctgctgtttgatcctcttggcaattacctggtgcacttctgcctatgggcctgaccaacgagctcagaagaaaggggacattatcctcggggggctctttcctattcattttggagtagcagccaaagatcaagatctaaagtcaaggccagagtctgtggaatgtatcaggtataatttccgtgggtttcgctggttacaagcaatgatatttgccatcgaggaaataaacagcagcccagtccttcttcccaacatgacactgggatacaggatatttgacacttgcaacactgtttctaaagccttggaggccactctgagttttgtggcacaaaataaaattgattctctgaacctcgacgagttctgcaactgctcagagcatatcccctctactatcgctgtggtgggagcaactggttcgggcatctccacagcggtggcaaacctgctgggcctcttctatattccccaggtcagctatgcctcctccagcagactcctcagcaacaaaaatcagttcaagtcctttctccgtaccatccccaatgatgaacaccaggccactgccatggcagacattatcgagtatttccgctggaactgggtgggcacaattgctgctgatgatgactacggccggccagggattgagaagtttcgagaggaagctgaggagagggacatctgcatcgacttcagtgaactcatctcccagtattctgatgaagaagagatccagcaagtggtggaggtgatccagaattccacagccaaagtcattgttgttttctctagtggcccagaccttgaaccccttatcaaggagattgtccggcgtaatatcacagggaggatctggctggccagcgaggcctgggccagctcttccttgattgccatgcccgagtacttccatgtggttggaggcaccattggattcgctctgaaggctggacagatcccaggtttccgggaattcctgcagaaagtccatcccagaaagtctgtccacaatggttttgccaaggagttttgggaagaaacctttaactgccacctccaagaaggtgctaaaggacctttagcactggacactttcctgagaggtcatgaagaaggtggtggcaggataagcaatagctccactgccttgcgacctctctgtacaggggacgagaacatcagcagcgtggagaccccttacatggattatacacatttacggatatcctacaatgtctacttagcggtctattccattgctcatgccctgcaagatatatatacatgcttacctggaagagggctcttcaccaatggttcctgcgcagatatcaagaaggttgaggcttggcaggtcctgaagcacctacggcacctaaactttaccaacaatatgggggagcaggtgactttcgatgaatgtggggacctggtggggaactattccatcatcaactggcacctctctccagaggatggctccatagtgtttaaggaagtcggatattacaacgtctatgccaagaaaggagaaaggctcttcatcaatgaggagaaaatcctgtggagtggattctccagggaggtacctttctccaactgcagtcgagactgcctggcagggacccggaaaggaatcattgagggggagcccacctgctgctttgagtgtgtggaatgtcctgatggggagtacagtgatgaaacagatgcaagtgcctgtgacaagtgccccgatgacttctggtccaatgagaaccacacttcttgcattgccaaggagattgagtttctgtcctggacggagccctttgggattgcactcactctctttgctgtgctgggcattttcctgacagccttcgtgctgggtgtcttcctcaagttccgtaacacacccattgtcaaggctaccaatcgagagctctcctacctcctcctcttctccttgctctgctgcttctccagctccctgttcttcattggtgagccccaggactggacatgccgcctgcgccagccagcctttggcatcagcttcgtgctctgcatatcatgcatcctagtgaaaaccaaccgtgtcctcctggtgtttgaggccaagatccccacgagcttccaccgcaagtggtgggggctcaacctgcagttcctgctggtcttcctctgcaccttcatgcagattgtcatctgtgtgatctggctctacactgcaccaccctcaagctaccgcaaccacgagctggaggatgagatcatctttatcacatgccacgagggctcgctcatggccctgggcttcttaattggctacacctgcctactggctgccatctgcttcttctttgccttcaagtcccggaagctgccagagaatttcaatgaagccaagttcatcaccttcagcatgctcatcttcttcatcgtctggatctccttcatcccagcctatgccagcacctatggcaagtttgtctctgccgtggaagtgatcgccatcctggcagccagctttggcttgctggcctgcatcttcttcaacaaggtctacatcatcctcttcaagccatcacgtaacaccatcgaggaggtgcgctgcagcactgctgcccatgctttcaaagtagcagcccgggccacgctgcgccgcagcaacgtctctcgcaagcggtccagcagccttgggggctccacgggatccacaccctcttcctccatcagcagtaagagcaacagtgaagaccccttcccacagcccgagaggcaaaagcagcagcagccactggccctgacccaacaagagcagcagccgcagccacagcagccctcgtccctacagcagcagccacagccacagccacagcccagatgcaagcagaaagtcattttcggcagtggcacagtcaccttctcactgagctttgatgagcctcagaagagtgccatggctcacaggaattctatgcaccagaactccctggaggcccagaaaagcaatgagaccctcaccagacaccaggcattactcccactacagtgcggggagacagactcagaactgagtgcccaggagagaggtcttcaagggcctgtagatggggacttccgaccagagatggaggaccctgaagagatgtccccagcgcttgtagtgtccagttcacaaagctttgtcatcagtggtggtggcagcactgtcacagaaaatatactgcattca